European Patent Application EP 4 538 371 A1, published April 16, 2025. Title: STRAINS AND METHOD FOR REDUCING THE PRODUCTION OF HYDROGEN SULFATE IN BEVERAGES. Applicant: Institut national de recherche pour l'agriculture, l'alimentation et l'environnement. Application EP. The sequence listing filed with the application follows.

SEQUENCE LISTING (9 sequences)

SEQ ID NO: 1 - DNA, 108 bp, Saccharomyces cerevisiae JN27
  source 1..108: mol_type = other DNA
atgggagaaattttagaactaactaataagaatttcatgagccacttgaaaaaggacataacttcgcaagaatccttgaaaagtagaattgaggataaaaaatggtga

SEQ ID NO: 2 - protein, 35 aa, Saccharomyces cerevisiae JN27
MGEILELTNKNFMSHLKKDITSQESLKSRIEDKKW

SEQ ID NO: 3 - DNA, 552 bp, Saccharomyces cerevisiae JN27
  source 1..552: mol_type = other DNA
atggatgtggtaccatctccgggtttaccagaaaaagtaaacgaaaaaagcaaaaatattcccttacctgaaggaattaaccttttatcatcaaaggagataatcgatctaattcaaacccacagacaccaattagagttatacgtcacaaaattcaatcccttaacggactttgctggaaagattcatgcattcagagatcaatttaaacaattggaagaaaattttgaagatttacatgagcaaaaagataaggtccaagccttattagaaaactgtaggattttagaatccaaatatgtagctagctggcaagattaccattccgaattttcaaaaaaatatggtgacatagcattaaaaaagaaattagaacaaaacacaaagaaacttgatgaggagagttcacagctagaaactaccacaaggtccattgactcagccgatgacctggatcagttcatcaaaaattatctggacatacgaacacaatatcacttgaggagagagaaactggcgacctgggataaacaaggtgatttgaaatactag

SEQ ID NO: 4 - protein, 183 aa, Saccharomyces cerevisiae JN27
MDVVPSPGLPEKVNEKSKNIPLPEGINLLSSKEIIDLIQTHRHQLELYVTKFNPLTDFAGKIHAFRDQFKQLEENFEDLHEQKDKVQALLENCRILESKYVASWQDYHSEFSKKYGDIALKKKLEQNTKKLDEESSQLETTTRSIDSADDLDQFIKNYLDIRTQYHLRREKLATWDKQGDLKY

SEQ ID NO: 5 - DNA, 1269 bp, Saccharomyces cerevisiae JN27
  source 1..1269: mol_type = other DNA
atggttgatcttatagcgagggatgactccgtagatacttgccaagcttctaacgactacaatgggcacgcaggtcttagaattctggcagtattcattatactgatatcgtcaggattgggagtttatttcccaattttgtcatcacggtattcgtttataaggctaccaaattggtgctttttcatagcgaagttcttcggttctggtgtcattgttgccacagcgttcgttcatcttctacagcccgcagccgaagctctgggagatgaatgtcttggtggcacatttgccgaatatccatgggcttttgggatctgtttaatgtcgcttttcttacttttcttcactgaaatcatcacgcattattttgtagcgaaaacgctgggacacgatcatggggaccatggggaagttaccagtattgatgttgatgctcccagttcgggatttgtcatcagaaatatggactcggatcctgtatctttcaataacgaagctgcctactccatccataatgacaaaactccgtacactactagaaatgaagagattgtcgctactcctataaaggaaaaagaacccggctcaaatgttactaattatgatctggaaccgggaaaaacagagtcactagctaatgaactagttccaaccagttcccatgcgacaaatctcgcttctgtacctggaaaagatcattattctcacgaaaatgaccatcaagatgtctcccagttggctacacgtatcgaggaggaagataaagagcagtatctcaatcagatactagctgtttttattctagaatttggcatcatctttcactctgtatttgtgggtctttcgctatctgtcgcgggtgaagaattcgaaaccttatttatcgttttaactttccaccaaatgttcgaaggtttgggtctaggcacaagagttgccgaaacgaattggccagaaagtgagaagtacacgccttggttaatgggattagccttcactttaacgtcacccatagcagtcgcggtaggtattggtgtcagacactcttggatacctggctctagaagagcattaattgctaatggtgtttttgactcgatatcatcaggaattcttatttatactggactagtcgaattaatggctcatgaattcttatactctaatcaattcaaaggacctgatggcctcaaaaaaatgcttagtgcatatctcatcatgtgttgtggagctgctttaatggctcttctagggaaatgggcatag

SEQ ID NO: 6 - protein, 422 aa, Saccharomyces cerevisiae JN27
MVDLIARDDSVDTCQASNDYNGHAGLRILAVFIILISSGLGVYFPILSSRYSFIRLPNWCFFIAKFFGSGVIVATAFVHLLQPAAEALGDECLGGTFAEYPWAFGICLMSLFLLFFTEIITHYFVAKTLGHDHGDHGEVTSIDVDAPSSGFVIRNMDSDPVSFNNEAAYSIHNDKTPYTTRNEEIVATPIKEKEPGSNVTNYDLEPGKTESLANELVPTSSHATNLASVPGKDHYSHENDHQDVSQLATRIEEEDKEQYLNQILAVFILEFGIIFHSVFVGLSLSVAGEEFETLFIVLTFHQMFEGLGLGTRVAETNWPESEKYTPWLMGLAFTLTSPIAVAVGIGVRHSWIPGSRRALIANGVFDSISSGILIYTGLVELMAHEFLYSNQFKGPDGLKKMLSAYLIMCCGAALMALLGKWA

SEQ ID NO: 7 - protein, 136 aa, Saccharomyces cerevisiae JN20
MGEILELTNKNFMSHLKKDITSQESLKSRIEDKNGDVASPKEDNYPLLNETAAWPDGVITSEEGCSSSGEKENSGLCSEESSEEDPEEAEEESARAFGELVAVLRDKDIPLNVLDEPQMKDWLEKYTGVYRSSWHG

SEQ ID NO: 8 - protein, 183 aa, Saccharomyces cerevisiae JN20
MDVVPSPGLPEKVNEKSKNIPLPEGINLLSSKEIIDLIQTHRHQLELYVTKFNPLTDFAGKIHAFRDQFKQLEENFEDLHEQKDKVQALLENCRILESKYVASWQDYHSEFSKKYGDIALKKKLEQNTKKLDGESSQLETTTRSIDSADDLDQFIKNYLDIRTQYHLRREKLATWDKQGNLKY

SEQ ID NO: 9 - protein, 422 aa, Saccharomyces cerevisiae JN20
MVDLIARDDSVDTCQASNGYNGHAGLRILAVFIILISSGLGVYFPILSSRYSFIRLPNWCFFIAKFFGSGVIVATAFVHLLQPAAEALGDECLGGTFAEYPWAFGICLMSLFLLFFTEIITHYFVAKTLGHDHGDHGEVTSIDVDAPSSGFVIRNMDSDPVSFNNEAAYSIHNDKTPYTTRNEEIVATPIKEKEPGSNVTNYDLEPGKTESLANELVPTSSHATNLASVPGKDHYSHENDHQDVSQLATRIEEEDKEQYLNQILAVFILEFGIIFHSVFVGLSLSVAGEEFETLFIVLTFHQMFEGLGLGTRVAETNWPESKKYMPWLMGLAFTLTSPIAVAVGIGVRHSWIPGSRRALIANGVFDSISSGILIYTGLVELMAHEFLYSNQFKGPDGLKKMLSAYLIMCCGAALMALLGKWA